European Patent Specification EP 3 769 785 B1, published June 26, 2024. Title: Agent for targeting heart comprising tannic acid. Applicant: Korea Research Institute of Chemical Technology Korea Advanced Institute of Science and Technology (KAIST). The sequence listing filed with the application follows.

SEQUENCE LISTING (2 sequences)

SEQ ID NO: 1 - protein, 154 aa, Artificial Sequence
  bFGF(basic fibroblast growth factor)
AAGSITTLPALPEDGGSGAFPPGHFKDPKRLYCKNGGFFLRIHPDGRVDGVREKSDPHIKLQLQAEERGVVSIKGVCANRYLAMKEDGRLLASKCVTDECFFFERLESNNYNTYRSRKYTSWYVALKRTGQYKLGSKTGPGQKAILFLPMSAKS

SEQ ID NO: 2 - protein, 11 aa, Artificial Sequence
  SP(substance P)
RPKPQQFFGLM